European Patent Application EP 4 442 703 A1, published October 9, 2024. Title: RECOMBINANT HUMANIZED COLLAGEN TYPE I ALPHA-1 (rhCol I a1A1), AND EXPRESSION VECTOR AND USE THEREOF. Applicant: SHANDONG D-NUTRIMEC BIOMEDICAL CO., LTD. The sequence listing filed with the application follows.

SEQUENCE LISTING (4 sequences)

SEQ ID NO: 1 - protein, 1060 aa, synthetic construct
  source 1..1060: note = rhCol1A1
GGSQLSYGYDEKSTGGISVPGPMGPSGPRGLPGPPGAPGPQGFQGPPGEPGEPGASGPMGPRGPPGPPGKNGDDGEAGKPGRPGERGPPGPQGARGLPGTAGLPGMKGHRGFSGLDGAKGDAGPAGPKGEPGSPGENGAPGQMGPRGLPGERGRPGAPGPAGARGNDGATGAAGPPGPTGPAGPPGFPGAVGAKGEAGPQGPRGSEGPQGVRGEPGPPGPAGAAGPAGNPGADGQPGAKGANGAPGIAGAPGFPGARGPSGPQGPGGPPGPKGNSGEPGAPGSKGDTGAKGEPGPVGVQGPPGPAGEEGKRGARGEPGPTGLPGPPGERGGPGSRGFPGADGVAGPKGPAGERGSPGPAGPKGSPGEAGRPGEAGLPGAKGLTGSPGSPGPDGKTGPPGPAGQDGRPGPPGPPGARGQAGVMGFPGPKGAAGEPGKAGERGVPGPPGAVGPAGKDGEAGAQGPPGPAGPAGERGEQGPAGSPGFQGLPGPAGPPGEAGKPGEQGVPGDLGAPGPSGARGERGFPGERGVQGPPGPAGPRGANGAPGNDGAKGDAGAPGAPGSQGAPGLQGMPGERGAAGLPGPKGDRGDAGPKGADGSPGKDGVRGLTGPIGPPGPAGAPGDKGESGPSGPAGPTGARGAPGDRGEPGPPGPAGFAGPPGADGQPGAKGEPGDAGAKGDAGPPGPAGPAGPPGPIGNVGAPGAKGARGSAGPPGATGFPGAAGRVGPPGPSGNAGPPGPPGPAGKEGGKGPRGETGPAGRPGEVGPPGPPGPAGEKGSPGADGPAGAPGTPGPQGIAGQRGVVGLPGQRGERGFPGLPGPSGEPGKQGPSGASGERGPPGPMGPPGLAGPPGESGREGAPGAEGSPGRDGSPGAKGDRGETGPAGPPGAPGAPGAPGPVGPAGKSGDRGETGPAGPAGPVGPVGARGPAGPQGPRGDKGETGEQGDRGIKGHRGFSGLQGPPGPPGSPGEQGPSGASGPAGPRGPPGSAGAPGKDGLNGLPGPIGPPGPRGRTGDAGPVGPPGPPGPPGPPGPPSAGFDFSFLPQPPQEKAHDGGRYYRA

SEQ ID NO: 2 - protein, 1057 aa, synthetic construct
  source 1..1057: note = amino acid sequence at positions 162 to 1,218 of the humanized collagen type I alpha 1 chain
QLSYGYDEKSTGGISVPGPMGPSGPRGLPGPPGAPGPQGFQGPPGEPGEPGASGPMGPRGPPGPPGKNGDDGEAGKPGRPGERGPPGPQGARGLPGTAGLPGMKGHRGFSGLDGAKGDAGPAGPKGEPGSPGENGAPGQMGPRGLPGERGRPGAPGPAGARGNDGATGAAGPPGPTGPAGPPGFPGAVGAKGEAGPQGPRGSEGPQGVRGEPGPPGPAGAAGPAGNPGADGQPGAKGANGAPGIAGAPGFPGARGPSGPQGPGGPPGPKGNSGEPGAPGSKGDTGAKGEPGPVGVQGPPGPAGEEGKRGARGEPGPTGLPGPPGERGGPGSRGFPGADGVAGPKGPAGERGSPGPAGPKGSPGEAGRPGEAGLPGAKGLTGSPGSPGPDGKTGPPGPAGQDGRPGPPGPPGARGQAGVMGFPGPKGAAGEPGKAGERGVPGPPGAVGPAGKDGEAGAQGPPGPAGPAGERGEQGPAGSPGFQGLPGPAGPPGEAGKPGEQGVPGDLGAPGPSGARGERGFPGERGVQGPPGPAGPRGANGAPGNDGAKGDAGAPGAPGSQGAPGLQGMPGERGAAGLPGPKGDRGDAGPKGADGSPGKDGVRGLTGPIGPPGPAGAPGDKGESGPSGPAGPTGARGAPGDRGEPGPPGPAGFAGPPGADGQPGAKGEPGDAGAKGDAGPPGPAGPAGPPGPIGNVGAPGAKGARGSAGPPGATGFPGAAGRVGPPGPSGNAGPPGPPGPAGKEGGKGPRGETGPAGRPGEVGPPGPPGPAGEKGSPGADGPAGAPGTPGPQGIAGQRGVVGLPGQRGERGFPGLPGPSGEPGKQGPSGASGERGPPGPMGPPGLAGPPGESGREGAPGAEGSPGRDGSPGAKGDRGETGPAGPPGAPGAPGAPGPVGPAGKSGDRGETGPAGPAGPVGPVGARGPAGPQGPRGDKGETGEQGDRGIKGHRGFSGLQGPPGPPGSPGEQGPSGASGPAGPRGPPGSAGAPGKDGLNGLPGPIGPPGPRGRTGDAGPVGPPGPPGPPGPPGPPSAGFDFSFLPQPPQEKAHDGGRYYRA

SEQ ID NO: 3 - DNA, 3171 bp, synthetic construct
  source 1..3171: mol_type = other DNA; note = DNA sequence encoding the amino acid sequence at positions 162 to 1,218 of the humanized collagen type I alpha 1 chain
cagctgtcttatggctatgatgagaaatcaaccggaggaatttccgtgcctggccccatgggtccctctggtcctcgtggtctccctggcccccctggtgcacctggtccccaaggcttccaaggtccccctggtgagcctggcgagcctggagcttcaggtcccatgggtccccgaggtcccccaggtccccctggaaagaatggagatgatggggaagctggaaaacctggtcgtcctggtgagcgtgggcctcctgggcctcagggtgctcgaggattgcccggaacagctggcctccctggaatgaagggacacagaggtttcagtggtttggatggtgccaagggagatgctggtcctgctggtcctaagggtgagcctggcagccctggtgaaaatggagctcctggtcagatgggcccccgtggcctgcctggtgagagaggtcgccctggagcccctggccctgctggtgctcgtggaaatgatggtgctactggtgctgccgggccccctggtcccaccggccccgctggtcctcctggcttccctggtgctgttggtgctaagggtgaagctggtccccaagggccccgaggctctgaaggtccccagggtgtgcgtggtgagcctggcccccctggccctgctggtgctgctggccctgctggaaaccctggtgctgatggacagcctggtgctaaaggtgccaatggtgctcctggtattgctggtgctcctggcttccctggtgcccgaggcccctctggaccccagggccccggcggccctcctggtcccaagggtaacagcggtgaacctggtgctcctggcagcaaaggagacactggtgctaagggagagcctggccctgttggtgttcaaggaccccctggccctgctggagaggaaggaaagcgaggagctcgaggtgaacccggacccactggcctgcccggaccccctggcgagcgtggtggacctggtagccgtggtttccctggcgcagatggtgttgctggtcccaagggtcccgctggtgaacgtggttctcctggccctgctggccccaaaggatctcctggtgaagctggtcgtcccggtgaagctggtctgcctggtgccaagggtctgactggaagccctggcagccctggtcctgatggcaaaactggcccccctggtcccgccggtcaagatggtcgccccggacccccaggcccacctggtgcccgtggtcaggctggtgtgatgggattccctggacctaaaggtgctgctggagagcccggcaaggctggagagcgaggtgttcccggaccccctggcgctgtcggtcctgctggcaaagatggagaggctggagctcagggaccccctggccctgctggtcccgctggcgagagaggtgaacaaggccctgctggctcccccggattccagggtctccctggtcctgctggtcctccaggtgaagcaggcaaacctggtgaacagggtgttcctggagaccttggcgcccctggcccctctggagcaagaggcgagagaggtttccctggcgagcgtggtgtgcaaggtccccctggtcctgctggtccccgaggggccaacggtgctcccggcaacgatggtgctaagggtgatgctggtgcccctggagctcccggtagccagggcgcccctggccttcagggaatgcctggtgaacgtggtgcagctggtcttccagggcctaagggtgacagaggtgatgctggtcccaaaggtgctgatggctctcctggcaaagatggcgtccgtggtctgaccggccccattggtcctcctggccctgctggtgcccctggtgacaagggtgaaagtggtcccagcggccctgctggtcccactggagctcgtggtgcccccggagaccgtggtgagcctggtccccccggccctgctggctttgctggcccccctggtgctgacggccaacctggtgctaaaggcgaacctggtgatgctggtgctaaaggcgatgctggtccccctggccctgccggacccgctggaccccctggccccattggtaatgttggtgctcctggagccaaaggtgctcgcggcagcgctggtccccctggtgctactggtttccctggtgctgctggccgagtcggtcctcctggcccctctggaaatgctggaccccctggccctcctggtcctgctggcaaagaaggcggcaaaggtccccgtggtgagactggccctgctggacgtcctggtgaagttggtccccctggtccccctggccctgctggcgagaaaggatcccctggtgctgatggtcctgctggtgctcctggtactcccgggcctcaaggtattgctggacagcgtggtgtggtcggcctgcctggtcagagaggagagagaggcttccctggtcttcctggcccctctggtgaacctggcaaacaaggtccctctggagcaagtggtgaacgtggtccccctggtcccatgggcccccctggattggctggaccccctggtgaatctggacgtgagggggctcctggtgccgaaggttcccctggacgagacggttctcctggcgccaagggtgaccgtggtgagaccggccccgctggaccccctggtgctcctggtgctcctggtgcccctggccccgttggccctgctggcaagagtggtgatcgtggtgagactggtcctgctggtcccgccggtcctgtcggccctgttggcgcccgtggccccgccggaccccaaggcccacgtggtgacaagggtgagacaggcgaacagggcgacagaggcataaagggtcaccgtggcttctctggcctccagggtccccctggccctcctggctctcctggtgaacaaggtccctctggagcctctggtcctgctggtccccgaggtccccctggctctgctggtgctcctggcaaagatggactcaacggtctccctggccccattgggccccctggtcctcgcggtcgcactggtgatgctggtcctgttggtccccccggccctcctggacctcctggtccccctggtcctcccagcgctggtttcgacttcagcttcctgccccagccacctcaagagaaggctcacgatggtggccgctactaccgggct

SEQ ID NO: 4 - DNA, 819 bp, synthetic construct
  source 1..819: mol_type = other DNA; note = DNA sequence encoding the amino acid sequence of the secretion signal peptide from T. cruzi alpha-mannosidase, the amino acid sequence of the GFP, and the sequence of TEV protease cleavage site
atgagactgctgaccgccctgttcgcctacttcatcgtggccctgatcctggccttcagcgtgtccgccaagagcatgcaccaccaccatcaccatcatcacatgagcaagggcgaggaactgttcaccggcgtggtgcccatcctggtggaactggacggcgacgtgaacggccacaagttctctgtgcggggcgagggcgagggggacgccacaaatggcaagctgaccctgaagttcatctgcaccaccggaaagctgcccgtgccctggcctaccctggtcacaaccctgacctacggcgtgcagtgcttcagcagataccccgaccacatgaagcggcacgatttcttcaagagcgccatgcccgagggctacgtgcaagaacggaccatcagcttcaaggacgacggcacctacaagaccagagccgaagtgaagttcgagggcgacaccctggtcaaccggatcgagctgaagggcatcgacttcaaagaggacggcaacatcctgggccacaagctggaatacaacttcaacagccacaacgtgtacatcaccgccgacaagcagaagaacggcatcaaggccaacttcaagatccggcacaacgtggaagatggcagcgtgcagctggccgaccactaccagcagaacacccccatcggcgacggccccgtgctgctgcccgacaatcactacctgagcacccagagcgtgctgagcaaggaccccaacgagaagcgggaccacatggtgctgctggaatttgtgaccgccgctggcatcacccacggcgagaacctgtacttccaaggg